European Patent Specification EP 4 010 500 B1, published February 19, 2025. Title: Bakterienstamm zur Freisetzung eines rekombinanten Proteins in einem Fermentationsverfahren. Applicant: Wacker Chemie AG Koch, Johanna Kujau, Marian. The sequence listing filed with the application follows.

SEQUENCE LISTING (7 sequences)

SEQ ID NO: 1 - DNA, 879 bp, Artificial Sequence
  DNS-Fragment xI
  misc_feature (1)..(879)
caattcgcgcgcgtaacaaaagtgtctataatcacggcagaaaagtccacattgattatttgcacggcgtcacactttgctatgccatagcatttttatccataagattagcggatcctacctgacgctttttatcgcaactctctactgtttctccatacccgtttttttgggctagaaataattttgtttaagaattctaaggaggaaattatatggtcaaatctcaaccgattttgagatatatcttgcgcgggattcccgcgattgcagtagcggttctgctttctgcatgtagtgcaaataacaccgcaaagaatatgcatcctgagacacgtgcagtgggtagtgaaacatcatcactgcaagcttctcaggatgaatttgaaaacctggttcgtaatgtcgacgtaaaatcgcgaattatggatcagtatgctgactggaaaggcgtacgttatcgtctgggcggcagcactaaaaaaggtatcgattgttctggtttcgtacagcgtacattccgtgagcaatttggcttagaacttccgcgttcgacttacgaacagcaggaaatgggtaaatctgtttcccgcagtaatttgcgtacgggtgatttagttctgttccgtgccggttcaacgggacgccatgtcggtatttatatcggcaacaatcagtttgtccatgcttccaccagcagtggtgttattatttccagcatgaatgaaccgtactggaagaagcgttacaacgaagcacgccgggttctcagccgcagctaagaattgcaagctggccgacgcgtcccacagccgccagttccgctggcggcattttaactttctttaatgaagccggaaaaatcccgcgcgcgaaggc

SEQ ID NO: 2 - DNA, 1131 bp, Artificial Sequence
  DNS-Fragment xII
  misc_feature (1)..(1131)
caattcgcgcgcgtaacaaaagtgtctataatcacggcagaaaagtccacattgattatttgcacggcgtcacactttgctatgccatagcatttttatccataagattagcggatcctacctgacgctttttatcgcaactctctactgtttctccatacccgtttttttgggctagaaataattttgtttaagaattctaaggaggaaattatatggcgcggataaaccgtatttcgatcacgctctgtgctttactttttaccaccctgcctttaacgcctatggcccatgcttcaaagcaagccagggagagttctgctaccactcatatcaccaaaaaagcagataaaaagaaaagcacggcaaccaccaaaaagacccagaaaacagcgaaaaaagccgccagtaaaagtacgaccaaaagcaaaaccgcttcttccgttaaaaaatcttccattaccgcttctaaaaacgccaaaactcgcagcaaacacgccgtcaataaaacggcctcagccagctttaccgaaaagtgtaccaaacgtaagggctataaatcgcattgtgtgaaagtcaaaaatgccgcgtcaggaactcttgccgacgcgcacaaagcgaaggtgcaaaaagctacgaaagtggcaatgaataaactgatgcagcaaattggtaagccatatcgttggggtggcagctcaccgcgtaccggttttgattgcagcggcctggtttattacgcttataaagatttggtgaaaattcgtattccgcgtacggcgaatgaaatgtatcacctgcgtgatgcagcgccaatcgaacgtagtgaactgaaaaacggcgacctggtctttttccgtactcagggacgcggcacagccgatcatgtcggcgtgtatgtcggcaacggcaaatttattcagtcaccgcgcacaggtcaggaaattcaaatcacttctctcagtgaagactactggcagcgccactatgttggcgctcgtcgggtaatgaccccaaaaacacttcgctaagaattgcaagctggccgacgcgctctcccacagccgccagttccgctggcggcattttaactttctttaatgaagccggaaaaatcccgcgcgcgaaggc

SEQ ID NO: 3 - DNA, 1599 bp, Artificial Sequence
  DNS-Fragment xIII
  misc_feature (1)..(1599)
acagaattctaaggaggaaattatatgaaaagaaaccgtttttttaatacctcggctgctattgccatttcgattgcattacagatcttttttccgtccgcttccgctttcgctcaggttcagctggtgcagagcggtgccgaagttgttaaaccgggtgcaagcgttaaactgagctgtaaagcaagcggctatatttttaccagctattatatgtattgggtgaaacaggcaccgggtcagggtctggaatggattggtgaaattaatccgagcaatggcgataccaattttaatgaaaaatttaaaagcaaagccaccctgaccgttgataaaagcgcaagcaccgcatatatggaactgagcagcctgcgtagcgaagataccgcagtttattattgtacccgtagtgatggtcgcaatgatatggatagctggggtcagggcaccctggtcaccgttagcagcgcaagcaccaaaggtccgagcgtttttccgctggcaccgagcagcaaaagcaccagcggtggcaccgcagcactgggttgtctggttaaagattattttccggaaccggttacagttagctggaatagcggtgcactgaccagtggtgttcatacctttccggcagttctgcaaagcagcggtctgtatagcctgagcagcgttgttaccgttccgagcagtagcctgggcacccagacctatatttgtaatgttaatcataaaccgagcaacaccaaagtggataaaaaagttgaaccgaaaagctgctaataaccatggagaaaataaagtgaaacaaagcactattgcactggcactcttaccgttactcttcacccctgttaccaaagccgatattgtgctcacccagagtccggcaaccctgagcgttagtccgggtgaacgtgcaaccattagctgtcgtgcaagccagcgtgttagcagcagcacctatagctatatgcattggtatcagcagaaaccgggtcagcctccgaaactgctgattaaatatgcaagcaatctggaaagcggtgttccggcacgttttagcggtagcggtagtggcaccgattttaccctgaccattagcagcgttgaaccggaagattttgccacctattattgtcagcatagctgggaaattcctccgacctttggtggtggcaccaaactcgagattaaacgtaccgttgcagcaccgagcgtgtttatctttccgcctagtgatgaacagctgaaaagcggcaccgcaagcgttgtttgtctgctgaataacttttatccgcgtgaagcaaaagttcagtggaaagttgataatgcactgcaaagcggtaatagccaagaaagcgttaccgaacaggatagcaaagatagcacctatagcctgtcaagcaccctgaccctgagcaaagcagattatgaaaaacacaaagtgtatgcctgcgaagttacccatcagggtctgagcagtccggttacaaaaagttttaatcgtggtgaatgtagctcttctgcccatcaccaccatcaccattaataagcttctagaagcttggctgttttggcggatgagagaagattttcgac

SEQ ID NO: 4 - DNA, 564 bp, Escherichia coli
  misc_feature (1)..(564): codierende DNS des Spr-Vorläufer-Proteins
atggtcaaatctcaaccgattttgagatatatcttgcgcgggattcccgcgattgcagtagcggttctgctttctgcatgtagtgcaaataacaccgcaaagaatatgcatcctgagacacgtgcagtgggtagtgaaacatcatcactgcaagcttctcaggatgaatttgaaaacctggttcgtaatgtcgacgtaaaatcgcgaattatggatcagtatgctgactggaaaggcgtacgttatcgtctgggcggcagcactaaaaaaggtatcgattgttctggtttcgtacagcgtacattccgtgagcaatttggcttagaacttccgcgttcgacttacgaacagcaggaaatgggtaaatctgtttcccgcagtaatttgcgtacgggtgatttagttctgttccgtgccggttcaacgggacgccatgtcggtatttatatcggcaacaatcagtttgtccatgcttccaccagcagtggtgttattatttccagcatgaatgaaccgtactggaagaagcgttacaacgaagcacgccgggttctcagccgcagc

SEQ ID NO: 5 - protein, 188 aa, Escherichia coli
  PEPTIDE (1)..(188): Aminosäuresequenz des Spr-Vorläufer-Proteins
MVKSQPILRYILRGIPAIAVAVLLSACSANNTAKNMHPETRAVGSETSSLQASQDEFENLVRNVDVKSRIMDQYADWKGVRYRLGGSTKKGIDCSGFVQRTFREQFGLELPRSTYEQQEMGKSVSRSNLRTGDLVLFRAGSTGRHVGIYIGNNQFVHASTSSGVIISSMNEPYWKKRYNEARRVLSRS

SEQ ID NO: 6 - DNA, 813 bp, Escherichia coli
  misc_feature (1)..(813): codierende DNS des Ydho-Vorläufer-Proteins
atggcgcggataaaccgtatttcgatcacgctctgtgctttactttttaccaccctgcctttaacgcctatggcccatgcttcaaagcaagccagggagagttctgctaccactcatatcaccaaaaaagcagataaaaagaaaagcacggcaaccaccaaaaagacccagaaaacagcgaaaaaagccgccagtaaaagtacgaccaaaagcaaaaccgcttcttccgttaaaaaatcttccattaccgcttctaaaaacgccaaaactcgcagcaaacacgccgtcaataaaacggcctcagccagctttaccgaaaagtgtaccaaacgtaagggctataaatcgcattgtgtgaaagtcaaaaatgccgcgtcaggaactcttgccgacgcgcacaaagcgaaggtgcaaaaagctacgaaagtggcaatgaataaactgatgcagcaaattggtaagccatatcgttggggtggcagctcaccgcgtaccggttttgattgcagcggcctggtttattacgcttataaagatttggtgaaaattcgtattccgcgtacggcgaatgaaatgtatcacctgcgtgatgcagcgccaatcgaacgtagtgaactgaaaaacggcgacctggtctttttccgtactcagggacgcggcacagccgatcatgtcggcgtgtatgtcggcaacggcaaatttattcagtcaccgcgcacaggtcaggaaattcaaatcacttctctcagtgaagactactggcagcgccactatgttggcgctcgtcgggtaatgaccccaaaaacacttcgc

SEQ ID NO: 7 - protein, 271 aa, Escherichia coli
  PEPTIDE (1)..(271): Aminosäuresequenz des Ydho-Vorläufer-Proteins
MARINRISITLCALLFTTLPLTPMAHASKQARESSATTHITKKADKKKSTATTKKTQKTAKKAASKSTTKSKTASSVKKSSITASKNAKTRSKHAVNKTASASFTEKCTKRKGYKSHCVKVKNAASGTLADAHKAKVQKATKVAMNKLMQQIGKPYRWGGSSPRTGFDCSGLVYYAYKDLVKIRIPRTANEMYHLRDAAPIERSELKNGDLVFFRTQGRGTADHVGVYVGNGKFIQSPRTGQEIQITSLSEDYWQRHYVGARRVMTPKTLR